European Patent Application EP 4 793 353 A1, published August 19, 2026. Title: Method for increasing heat-stress-tolerance of pollen grains. Applicant: PLANTIK BIOSCIENCES. Application EP. The sequence listing filed with the application follows.

SEQUENCE LISTING (25 sequences)

SEQ ID NO: 1 - DNA, 244 bp, Solanum lycopersicum
  source 1..244: mol_type = genomic DNA
tcatataaatttatatcagatcgtaattttcaaaacatgccatatgtatcgataggagaaaattaaaaaataataagttataaattaaactcataaaatttaaattttaaatgccggtggcctatacggagacgctataattgacagctaaagccactggtatttgctgtatccaaaaaaataattcagacgtcattttctctgtcattaatcttattacactattgtgtccaattccaaaaat

SEQ ID NO: 2 - DNA, 1247 bp, Solanum lycopersicum
  source 1..1247: mol_type = genomic DNA
aattgacttagttataactatttaaaaaaaacactaattcaatcataatatattagtaattgacttcatacttggttacaaacattaaaataaaaaaaccagttcaatcataatataataattgacatcaatattcttgtctccttaatcaacatcattagtgttccttgaacacaataattaaaaattatgtactacaagtgaaatatacataaataatgatttaaaataatagtgaaaatgaggataagtgcaaacgtggcaaaagaatttagcagtatttgatccacaaggtgcaaagggtccataggaatagaaaagaagatttcatacagctaggctgcacgtatcattttttcctaaattcacttgatttattttcctttctagttaaaaaaaaatgacacttttttatatttaatattttttctattttaattcattgtttgatctatttttatttttaatcaatttaaaaaagaatcattatattctttttttagcaactttataatttcaatctactcctttgaaaatcttcttacctttcttacacgttgtgttaaatcaaaataggtcactcaatttaaaacgaaagaatcatattcttaatgaaatgatttataggtcactcacatttccggtctgtttccttcttattattcttgaataagtgaaacaacggccacagagtttttttccctgacttggtttgttttcccattataaaattttggtgtttcttctttttctgaacctaaaaggtttgatttttttattcttctttgcttcatttcttttcttagtcatattatgttgattttagaaatggggtttaaaaaagagtgattttttaagccattcttgacttgttctgtttgtgttgtgtgcaggtttttggttatttaacttctttgtttccttctttctgtaaggtataataaggcaaaatctttctttctgtttctgagggttttcttgtttgggggtggggtgggggaggacaagtaaggaaaagtagaggaactattgaagttttgaagagttatgtcatgcttgtctatatttagtttcctttttgctctattttatatgatcaagaaattcactttttcttgatatagaaaaatcattttttttaaaacccccttttgactattaagtattgaatttgatgattttgagattgccttttactgtgtgcctaaacatactgttttttttcttgatatgcagtagttttagcc

SEQ ID NO: 3 - DNA, 11 bp, Solanum lycopersicum
  source 1..11: mol_type = genomic DNA
taattcagacg

SEQ ID NO: 4 - DNA, 819 bp, Solanum lycopersicum
  source 1..819: mol_type = genomic DNA
ttttcaaaacatgccatatgtatcgataggagaaaattaaaaaataataagttataaattaaactcataaaatttaaattttaaatgccggtggcctatacggagacgctataattgacagctaaagccactggtatttgctgtatccaaaaaaatcattttctctgtcattaatcttatattgtgtccaattccaaaaatgatgctcacatttcctgtctgtttccttcttattattcttgaataagtgaaacaacggccacagagtttttttccctgacttggtttgttttcccattataaaattttggtgtttcttctttttctgaacctaaaaggttggattttttaatcctcttgcttcatttcttttcttagtcatattatgttgattttagaaatggggtttaaaaaagagtgattttttaagccattcttgacttgttctgtttgggttgggtgcaggtttttggttatttaacttctttgtttcctcctttctggaagggtttataaggcaaaatctttctttctgtttctgagggttttcttgtttgggggtggggtgggggaggacaagtaaggaaaagtagaggaactattgaagttttgaagagttatgtcatgcttgtctatatttagtttcctttttgctctattttatatgatcaagaaattcactttttcttgatatagaaaaatcattttttttaaaacccccttttgactattaagtattgaatttgatgattttgagattgccttttactgtgtgcctaaacatactgttttttttcttgatatgcagtagttttagcc

SEQ ID NO: 5 - DNA, 988 bp, Solanum lycopersicum
  source 1..988: mol_type = genomic DNA
taatttcaatctactcctttgaaaccattaaaatcttcttacctttcttacacgttgtgttaaatcaaaataggtcactcaatttaaaacaaaagaatcatattcttaatgaaatgatttatagtcatataaatttatatcagatcgtaattttcaaaacatgccatatgtatcgataggagaaaattaaaaaataataagttataaattaaactcataaaatttaaattttaaatgccggtggcctatacggagacgctataattgacagctaaagccactggtatttgctgtatccaaaaaaataattcagacgtcattttctctgtcattaatcttattacactattgtgtccaattccaaaaatgatgctcacatttcccgtctgtttccttcttattattcttgaataagtgaaacaacggccacagagtttttttccctgacttggtttgttttcccattataaaattttggtgtttcttctttttctgaacctaaaaggtttgatttttttattcttctttgcttcatttcttttcttagtcatattatgttgattttagaaatggggtttaaaaaagagtgattttttaagccattcttgacttgttctgtttgtgttgtgtgcaggtttttggttatttaacttctttgtttccttctttctgtaaggtataataaggcaaaatctttctttctgtttctgagggttttcttgtttgggggtggggtgggggaggacaagtaaggaaaagtagaggaactattgaagttttgaagagttatgtcatgcttgtctatatttagtttcctttttgctctattttatatgatcaagaaattcactttttcttgatatagaaaaatcattttttttaaaacccccttttgactattaagtattgaatttgatgattttgagattgccttttactgtgtgcctaaacatactgttttttttcttgatatgcagtagttttagcc

SEQ ID NO: 6 - DNA, 359 bp, Solanum lycopersicum
  source 1..359: mol_type = genomic DNA
tcaatctactcctttgaaaccattaaaatcttcttacctttcttacacgttgtgttaaatcaaaataggtcactcaatttaaaacaaaagaatcatattcttaatgaaatgatttatagtcatataaatttatatcagatcgtaattttcaaaacatgccatatgtatcgataggagaaaattaaaaaataataagttataaattaaactcataaaatttaaattttaaatgccggtggcctatacggagacgctataattgacagctaaagccactggtatttgctgtatccaaaaaaataattcagacgtcattttctctgtcattaatcttattacactattgtgtccaattccaa

SEQ ID NO: 7 - DNA, 326 bp, Solanum lycopersicum
  source 1..326: mol_type = genomic DNA
tcaatctactcctttgcttcttacctttcttacacgttgtgttaaatcaaaataggtcactcaatttaaaacgaaagaatcatattcttaatgaaatgatttatagtcatataaatttatatcagatcgtaattttcaaaacatgccatatgtatcgataggagaaaattaaaaaataataagttataaattaaactcataaaatttaaattttaaatgccggtggcctatacggagacgctataattgacagctaaagccactggtatttgctgtatccaaagacgtcattttctctgtcattaatcttatgtgtccaattccaa

SEQ ID NO: 8 - DNA, 63 bp, Solanum lycopersicum
  source 1..63: mol_type = genomic DNA
cactggtatttgctgtatccaaaaaaaacgtcattttctctgtcatattgtgtccaattccaa

SEQ ID NO: 9 - DNA, 111 bp, Solanum lycopersicum
  source 1..111: mol_type = genomic DNA
tcaatctactcctttgaaaatcttcttacctttcttacacgttgtgttaaatcaaaataggtcactcaatttaaaacgaaagaatcatattcttaatgaaatgatttatag

SEQ ID NO: 10 - DNA, 257 bp, Solanum lycopersicum
  source 1..257: mol_type = genomic DNA
tcaatctactcctttgaaaaatcttcttacctttcttacacgttgtgttaaatcaaaataggtcactcaatttaaaacgaaagaatcatattcttaatgaaaagttataaattaaactcataaaatttaaattttaaatgccggtggcctatacggagacgctataattgacagctaaagccactggtatttgctgtatccaaaaaaattcagacgtcattttctctgtcattaatctttattgtgtccaattccaa

SEQ ID NO: 11 - DNA, 333 bp, Solanum lycopersicum
  source 1..333: mol_type = genomic DNA
atgatttatagtcatataaatttatatcagatcgtaattttcaaaacatgccatatgtatcgataggagaaaattaaaaaataataagttataaattaaactcataaaatttaaattttaaatgccggtggcctatacggagacgctataattgacagctaaagccactggtatttgctgtatccaaaaaaataattcagacgtcattttctctgtcattaatcttattacactattgtgtccaattccaaaaatgatgctcacatttcccgtctgtttccttcttattattcttgaataagtgaaacaacggccacagagtttttttccctg

SEQ ID NO: 12 - DNA, 71 bp, Solanum lycopersicum
  source 1..71: mol_type = genomic DNA
tatttgctgtatccaaaaaaataattcagacgtcattttctctgtcattaatcttattacactattgtgtc

SEQ ID NO: 13 - DNA, 54 bp, Solanum lycopersicum
  source 1..54: mol_type = genomic DNA
tatttgctgtatccaaaaaaatcattttctctgtcattaatcttatattgtgtc

SEQ ID NO: 14 - DNA, 58 bp, Solanum lycopersicum
  source 1..58: mol_type = genomic DNA
tatttgctgtatccaaaaaaatcgtcattttctctgtcattaatcttattattgtgtc

SEQ ID NO: 15 - DNA, 47 bp, Solanum lycopersicum
  source 1..47: mol_type = genomic DNA
tattcgtgtatcaaaaaaatatacaaactttgtattaatattaagat

SEQ ID NO: 16 - DNA, 21 bp, synthetic construct
  source 1..21: mol_type = other DNA
aatctactcctttgaaaccat

SEQ ID NO: 17 - DNA, 21 bp, synthetic construct
  source 1..21: mol_type = other DNA
atggtttcaaaggagtagatt

SEQ ID NO: 18 - DNA, 21 bp, synthetic construct
  source 1..21: mol_type = other DNA
aaaattacgatctgatataaa

SEQ ID NO: 19 - DNA, 21 bp, synthetic construct
  source 1..21: mol_type = other DNA
tttatatcagatcgtaatttt

SEQ ID NO: 20 - DNA, 21 bp, synthetic construct
  source 1..21: mol_type = other DNA
ctgtatccaaaaaaataattc

SEQ ID NO: 21 - DNA, 21 bp, synthetic construct
  source 1..21: mol_type = other DNA
gaattatttttttggatacag

SEQ ID NO: 22 - DNA, 21 bp, synthetic construct
  source 1..21: mol_type = other DNA
gaattggacacaatagtgtaa

SEQ ID NO: 23 - DNA, 21 bp, synthetic construct
  source 1..21: mol_type = other DNA
ttacactattgtgtccaattc

SEQ ID NO: 24 - DNA, 28 bp, synthetic construct
  source 1..28: mol_type = other DNA
catctgaaaagtgaatctatcattgaca

SEQ ID NO: 25 - DNA, 28 bp, synthetic construct
  source 1..28: mol_type = other DNA
ggctaaaactactgcatatcaagaaaaa